European Patent Specification EP 3 810 201 B9, published August 2, 2023. Title: GIP/GLP1 AGONIST COMPOSITIONS. Applicant: Eli Lilly and Company. Application PCT/US2019/037146. The sequence listing filed with the application follows.

SEQUENCE LISTING (1 sequence)

SEQ ID NO: 1 - protein, 39 aa, Artificial Sequence
  Synthetic Construct
  MISC_FEATURE (2)..(2): Xaa at position 2 is nonnaturally occurring amino acid 2-Aminoisobutyric Acid
  MISC_FEATURE (13)..(13): Xaa at position 13 is nonnaturally occurring amino acid 2-Aminoisobutyric Acid
  MOD_RES (20)..(20): Lys at position 20 is chemically modified through conjugation to the epsilon-amino group of the K side-chain with (2-[2-(2-Amino-ethoxy)-ethoxy]-acetyl)2-(gamma-Glu)1-CO-(CH2)18-C O2H
  MOD_RES (39)..(39): Ser at position 39 is amidated as a C-terminal primary amide
YXEGTFTSDYSIXLDKIAQKAFVQWLIAGGPSSGAPPPS